European Patent Application EP 4 556 562 A1, published May 21, 2025. Title: Mutant microorganism of Corynebacterium genus producing L-glutamic acid and method for producing L-glutamic acid using the same. Applicant: DAESANG CORPORATION. The sequence listing filed with the application follows.

SEQUENCE LISTING (9 sequences)

SEQ ID NO: 1 - DNA, 674 bp, synthetic construct
  source 1..674: mol_type = other DNA
atggatatgacgatctcccgcgccaccatggcccaaatccttgactacaccctcctcggaccagaagtaaccaactccgaactggccgcatttatagattccgcaattgagctgggagtcggaacgatctgtgtccccaatagcatggtcaacttaactgcaaaagcccaagaagctggaattcgcgtggccaccgtcgcaggattcccgcacggcaaaaccccgcgttggtgaaagccgccgaagctcgccttgccgtacagtccggagcttccgaagtagatgttgttttggatattgcggtagtgaaagagggagatgccaataggttgctgcaggaaattgtggcaatcagggaggctgttccatctcctgtggtgctgaaattcatcctcgagacggctgtcgtgggtgatgatgcaattgtgactgcagtgaatgcattgattgctgcaggtgctgacttcgctaaaacttccacgggattccacccagcgggaggagcaactgttgaggctgttcgggtgatggcttcggcttctcggggaagggttggaattaaggctgccggtggggtgaacacttgggaagatgcggtggcgtttgttgaagcaggggctactcgcattggaacttctaatgcgggagccattttggagggtgcgccggagtag

SEQ ID NO: 2 - protein, 214 aa, synthetic construct
MDMTISRATMAQILDYTLLGPEVTNSELAAFIDSAIELGVGTICVPNSMVNLTAKAQEAGIRVATVAGFPHGKTPRWKPPKLALPYSPELPKMLFWILRKREMPIGCCRKLWQSGRLFHLLWCNSSSRRLSWVMMQLLQMHLLQVLTSLKLPRDSTQREEQLLRLFGWLRLLGEGLELRLPVGTLGKMRWRLLKQGLLALELLMREPFWRVRRS

SEQ ID NO: 3 - DNA, 675 bp, Corynebacterium sp.
  source 1..675: mol_type = genomic DNA
atggatatgacgatctcccgcgccaccatggcccaaatccttgactacaccctcctcggaccagaagtaaccaactccgaactggccgcatttatagattccgcaattgagctgggagtcggaacgatctgtgtccccaatagcatggtcaacttaactgcaaaagcccaagaagctggaattcgcgtggccaccgtcgcaggattcccgcacggcaaaacccccgcgttggtgaaagccgccgaagctcgccttgccgtacagtccggagcttccgaagtagatgttgttttggatattgcggtagtgaaagagggagatgccaataggttgctgcaggaaattgtggcaatcagggaggctgttccatctcctgtggtgctgaaattcatcctcgagacggctgtcgtgggtgatgatgcaattgtgactgcagtgaatgcattgattgctgcaggtgctgacttcgctaaaacttccacgggattccacccagcgggaggagcaactgttgaggctgttcgggtgatggcttcggcttctcggggaagggttggaattaaggctgccggtggggtgaacacttgggaagatgcggtggcgtttgttgaagcaggggctactcgcattggaacttctaatgcgggagccattttggagggtgcgccggagtag

SEQ ID NO: 4 - protein, 224 aa, Corynebacterium sp.
MDMTISRATMAQILDYTLLGPEVTNSELAAFIDSAIELGVGTICVPNSMVNLTAKAQEAGIRVATVAGFPHGKTPALVKAAEARLAVQSGASEVDVVLDIAVVKEGDANRLLQEIVAIREAVPSPVVLKFILETAVVGDDAIVTAVNALIAAGADFAKTSTGFHPAGGATVEAVRVMASASRGRVGIKAAGGVNTWEDAVAFVEAGATRIGTSNAGAILEGAPE

SEQ ID NO: 5 - DNA, 5719 bp, synthetic construct
  source 1..5719: mol_type = other DNA
tgccgcaagcactcagggcgcaagggctgctaaaggaagcggaacacgtagaaagccagtccgcagaaacggtgctgaccccggatgaatgtcagctactgggctatctggacaagggaaaacgcaagcgcaaagagaaagcaggtagcttgcagtgggcttacatggcgatagctagactgggcggttttatggacagcaagcgaaccggaattgccagctggggcgccctctggtaaggttgggaagccctgcaaagtaaactggatggctttcttgccgccaaggatctgatggcgcaggggatcaagatctgatcaagagacaggatgaggatcgtttcgcatgattgaacaagatggattgcacgcaggttctccggccgcttgggtggagaggctattcggctatgactgggcacaacagacaatcggctgctctgatgccgccgtgttccggctgtcagcgcaggggcgcccggttctttttgtcaagaccgacctgtccggtgccctgaatgaactccaagacgaggcagcgcggctatcgtggctggccacgacgggcgttccttgcgcagctgtgctcgacgttgtcactgaagcgggaagggactggctgctattgggcgaagtgccggggcaggatctcctgtcatctcaccttgctcctgccgagaaagtatccatcatggctgatgcaatgcggcggctgcatacgcttgatccggctacctgcccattcgaccaccaagcgaaacatcgcatcgagcgagcacgtactcggatggaagccggtcttgtcgatcaggatgatctggacgaagagcatcaggggctcgcgccagccgaactgttcgccaggctcaaggcgcggatgcccgacggcgaggatctcgtcgtgacccatggcgatgcctgcttgccgaatatcatggtggaaaatggccgcttttctggattcatcgactgtggccggctgggtgtggcggaccgctatcaggacatagcgttggctacccgtgatattgctgaagagcttggcggcgaatgggctgaccgcttcctcgtgctttacggtatcgccgctcccgattcgcagcgcatcgccttctatcgccttcttgacgagttcttctgagcgggactctggggttcgctagaggatcgatcctttttaacccatcacatatacctgccgttcactattatttagtgaaatgagatattatgatattttctgaattgtgattaaaaaggcaactttatgcccatgcaacagaaactataaaaaatacagagaatgaaaagaaacagatagattttttagttctttaggcccgtagtctgcaaatccttttatgattttctatcaaacaaaagaggaaaatagaccagttgcaatccaaacgagagtctaatagaatgaggtcgaaaagtaaatcgcgcgggtttgttactgataaagcaggcaagacctaaaatgtgtaaagggcaaagtgtatactttggcgtcaccccttacatattttaggtctttttttattgtgcgtaactaacttgccatcttcaaacaggagggctggaagaagcagaccgctaacacagtacataaaaaaggagacatgaacgatgaacatcaaaaagtttgcaaaacaagcaacagtattaacctttactaccgcactgctggcaggaggcgcaactcaagcgtttgcgaaagaaacgaaccaaaagccatataaggaaacatacggcatttcccatattacacgccatgatatgctgcaaatccctgaacagcaaaaaaatgaaaaatatcaagtttctgaatttgattcgtccacaattaaaaatatctcttctgcaaaaggcctggacgtttgggacagctggccattacaaaacgctgacggcactgtcgcaaactatcacggctaccacatcgtctttgcattagccggagatcctaaaaatgcggatgacacatcgatttacatgttctatcaaaaagtcggcgaaacttctattgacagctggaaaaacgctggccgcgtctttaaagacagcgacaaattcgatgcaaatgattctatcctaaaagaccaaacacaagaatggtcaggttcagccacatttacatctgacggaaaaatccgtttattctacactgatttctccggtaaacattacggcaaacaaacactgacaactgcacaagttaacgtatcagcatcagacagctctttgaacatcaacggtgtagaggattataaatcaatctttgacggtgacggaaaaacgtatcaaaatgtacagcagttcatcgatgaaggcaactacagctcaggcgacaaccatacgctgagagatcctcactacgtagaagataaaggccacaaatacttagtatttgaagcaaacactggaactgaagatggctaccaaggcgaagaatctttatttaacaaagcatactatggcaaaagcacatcattcttccgtcaagaaagtcaaaaacttctgcaaagcgataaaaaacgcacggctgagttagcaaacggcgctctcggtatgattgagctaaacgatgattacacactgaaaaaagtgatgaaaccgctgattgcatctaacacagtaacagatgaaattgaacgcgcgaacgtctttaaaatgaacggcaaatggtacctgttcactgactcccgcggatcaaaaatgacgattgacggcattacgtctaacgatatttacatgcttggttatgtttctaattctttaactggcccatacaagccgctgaacaaaactggccttgtgttaaaaatggatcttgatcctaacgatgtaacctttacttactcacacttcgctgtacctcaagcgaaaggaaacaatgtcgtgattacaagctatatgacaaacagaggattctacgcagacaaacaatcaacgtttgcgccgagcttcctgctgaacatcaaaggcaagaaaacatctgttgtcaaagacagcatccttgaacaaggacaattaacagttaacaaataaaaacgcaaaagaaaatgccgatgggtaccgagcgaaatgaccgaccaagcgacgcccaacctgccatcacgagatttcgattccaccgccgccttctatgaaaggttgggcttcggaatcgttttccgggacgccctcgcggacgtgctcatagtccacgacgcccgtgattttgtagccctggccgacggccagcaggtaggccgacaggctcatgccggccgccgccgccttttcctcaatcgctcttcgttcgtctggaaggcagtacaccttgataggtgggctgcccttcctggttggcttggtttcatcagccatccgcttgccctcatctgttacgccggcggtagccggccagcctcgcagagcaggattcccgttgagcaccgccaggtgcgaataagggacagtgaagaaggaacacccgctcgcgggtgggcctacttcacctatcctgcccggctgacgccgttggatacaccaaggaaagtctacacgaaccctttggcaaaatcctgtatatcgtgcgaaaaaggatggatataccgaaaaaatcgctataatgaccccgaagcagggttatgcagcggaaaagcgctgcttccctgctgttttgtggaatatctaccgactggaaacaggcaaatgcaggaaattactgaactgaggggacaggcgagagacgatgccaaagagctcctgaaaatctcgataactcaaaaaatacgcccggtagtgatcttatttcattatggtgaaagttggaacctcttacgtgccgatcaacgtctcattttcgccaaaagttggcccagggcttcccggtatcaacagggacaccaggatttatttattctgcgaagtgatcttccgtcacaggtatttattcggcgcaaagtgcgtcgggtgatgctgccaacttactgatttagtgtatgatggtgtttttgaggtgctccagtggcttctgtttctatcagctcctgaaaatctcgataactcaaaaaatacgcccggtagtgatcttatttcattatggtgaaagttggaacctcttacgtgccgatcaacgtctcattttcgccaaaagttggcccagggcttcccggtatcaacagggacaccaggatttatttattctgcgaagtgatcttccgtcacaggtatttattcggcgcaaagtgcgtcgggtgatgctgccaacttactgatttagtgtatgatggtgtttttgaggtgctccagtggcttctgtttctatcagggctggatgatcctccagcgcggggatctcatgctggagttcttcgcccaccccaaaaggatctaggtgaagatcctttttgataatctcatgaccaaaatcccttaacgtgagttttcgttccactgagcgtcagaccccgtagaaaagatcaaaggatcttcttgagatcctttttttctgcgcgtaatctgctgcttgcaaacaaaaaaaccaccgctaccagcggtggtttgtttgccggatcaagagctaccaactctttttccgaaggtaactggcttcagcagagcgcagataccaaatactgttcttctagtgtagccgtagttaggccaccacttcaagaactctgtagcaccgcctacatacctcgctctgctaatcctgttaccagtggctgctgccagtggcgataagtcgtgtcttaccgggttggactcaagacgatagttaccggataaggcgcagcggtcgggctgaacggggggttcgtgcacacagcccagcttggagcgaacgacctacaccgaactgagatacctacagcgtgagctatgagaaagcgccacgcttcccgaagggagaaaggcggacaggtatccggtaagcggcagggtcggaacaggagagcgcacgagggagcttccagggggaaacgcctggtatctttatagtcctgtcgggtttcgccacctctgacttgagcgtcgatttttgtgatgctcgtcaggggggcggagcctatggaaaaacgccagcaacgcggcctttttacggttcctggccttttgctggccttttgctcacatgttctttcctgcgttatcccctgattctgtggataaccgtattaccgcctttgagtgagctgataccgctcgccgcagccgaacgaccgagcgcagcgagtcagtgagcgaggaagcggaagagcgcccaatacgcaaaccgcctctccccgcgcgttggccgattcattaatgcagctggcacgacaggtttcccgactggaaagcgggcagtgagcgcaacgcaattaatgtgagttagctcactcattaggcaccccaggctttacactttatgcttccggctcgtatgttgtgtggaattgtgagcggataacaatttcacacaggaaacagctatgacatgattacgccaagcttgcatgcctgcaggtcgactctagaggatccccgggtaccgagctcgaattcactggccgtcgttttacaacgtcgtgactgggaaaaccctggcgttacccaacttaatcgccttgcagcacatccccctttcgccagctggcgtaatagcgaagaggcccgcaccgatcgcccttcccaacagttgcgcagcctgaatggcgaatggcgataagctagcttcacgc

SEQ ID NO: 6 - DNA, 21 bp, synthetic construct
  source 1..21: mol_type = other DNA
cgacctggtcaaacgccttcc

SEQ ID NO: 7 - DNA, 19 bp, synthetic construct
  source 1..19: mol_type = other DNA
tcaccaacgcggggttttg

SEQ ID NO: 8 - DNA, 20 bp, synthetic construct
  source 1..20: mol_type = other DNA
gcaaaaccccgcgttggtga

SEQ ID NO: 9 - DNA, 20 bp, synthetic construct
  source 1..20: mol_type = other DNA
gtcacttcccccgcttcagg